European Patent Application EP 4 685 226 A1, published January 28, 2026. Title: NOVEL PREVOTELLA MERDAE IMMUNOACTIS STRAIN AND USE THEREOF. Applicant: THE ASAN FOUNDATION. Application EP. The sequence listing filed with the application follows.

SEQUENCE LISTING (1 sequence)

SEQ ID NO: 1 - DNA, 1026 bp, synthetic construct
  source 1..1026: mol_type = other DNA
aaggatggggatgcgtctgattagcttgttggcggggtaacggcccaccaaggcgacgatcagtaggggttctgagaggaaggtcccccacattggaactgagacacggtccaaactcctacgggaggcagcagtgaggaatattggtcaatggacggaagtctgaaccagccaagtagcgtgcaggaagacggccctatgggttgtaaactgcttttatacggggataaagtgagccacgtgtggcttattgcaggtaccgtatgaataaggaccggctaattccgtgccagcagccgcggtaatacggaaggtccgggcgttatccggatttattgggtttaaagggagcgtaggccgtttgttaagcgtgttgtgaaatgtcggggctcaacctgggcattgcagcgcgaactggcagacttgagtgcgcgggaagtaggcggaattcgtcgtgtagcggtgaaatgcttagatatgacgaagaactccgattgcgaaggcagcctgctgtagcgtaactgacgctgaagctcgaaagcgtgggtatcgaacaggattagataccctggtagtccacgcggtaaacgatggatgctcgctgtttgcgtctgacgtaagcggccaagcgaaagcgttaagcatcccacctggggagtacgccggcaacggtgaaactcaaaggaattgacgggggcccgcacaagcggaggaacatgtggtttaattcgatgatacgcgaggaaccttacccgggcttgaactgcaggcgaacgattcagagatgatgaggcccttcggggcgcctgtggaggtgctgcatggttgtcgtcagctcgtgccgtgaggtgtcggcttaagtgccataacgagcgcaacccttgctctcagttgccatcggttaaagccgggcactctgtgaggactgcctccgcaaggagtgaggaaggtggggatgacgtcaaatcagcacggcccttacgtccggggctacacacgtgttacaatggcatgtacagaaagctg